European Patent Application EP 4 692 363 A1, published February 11, 2026. Title: Method for producing methyl compound. Applicant: Mitsubishi Chemical Corporation. Application WO. The sequence listing filed with the application follows.

SEQUENCE LISTING (10 sequences)

SEQ ID NO: 1 - DNA, 1109 bp, synthetic construct
  source 1..1109: mol_type = other DNA
catatgacaatatcactagaaaatacgactgtaggccagaatccggccggtggccctccgaccggaaaagcaccgctggacatggaaggcttggcgtggattttgtttggtgctagcgcattccaatatctgaatgcagcgtgcgaattgaacctgttcgagttgctggagaacaaaccgggtttgacgaagccacaaatcggtgctgaactgggtctcgctgatcgtgcaaatgacatcctgctgcttggtgccactgcgaccggtatgctgacggtggaagatggtcgctaccagctggcgacggtcctggctgagttgctgaagaccgatgattggcagcgttttaaagataccgtgggttttgaacaatacgtttgctacgagggccagatcgatttcaccgagagcctacgctctaactccaatgttggtctgcgccgcgtgcgcggcagcggtcgtgatctgtatcatcgtttacatgaaaacccgcaaatggaacaggcgttctacaagtacatgcgttcttggtcagaactggcgaaccagcatctggtggaagttctggatctgagcggtacgagcaaactgctggactgtggtggtggcgacgcagttaattcgattgcattggcccaggcgaacccgcacattgaagcgggtattctggagatcccgccaactgcgccactgaccgaaaaaaaaatcgcggaggcaggcttatctgatcgtattaccgtaaagccgggagacatgcacaccgatgaatttccgaccggctatgacaccgtgatgttcgcacaccagctggtcatctggactccggaggagaataccgccttgctgcgtaaagcgtataacgcacttccggaaggcggccgtgttattatctttaactccatgtccaacgacgagggcgacggcccggttgtggccgcgctcgacagcgtttatttcgccgcgctgccggctgaaggtggcatgatttacagctgggctacctacgaggagagcctaacgaaggcgggtttcaacccggagacatttcaacgtatcgacttcccgggttggaccccgcacggcgtgatcatcgcgaccaagtaagatct

SEQ ID NO: 2 - DNA, 3222 bp, synthetic construct
  source 1..3222: mol_type = other DNA
catatgccctcagatattgaaatagctagggcagctaccctcaagcccatcgcacaggtcgcagagaagctgggcattccggatgaagcgctgcacaactacggcaagcacatcgcgaaaattgaccacgatttcatcgcctctctggagggtaagccggaaggcaagttggttctggttaccgctataagcccgaccccggctggcgagggcaagaccacgaccaccgttggattgggtgatgcgctgaatcgtattggtaagcgcgcggtgatgtgcctgcgcgaaccgagcctgggtccgtgctttggtatgaaaggtggagcggctggtggcggcaaagcacaagttgtgccgatggaacagatcaaccttcacttcaccggcgacttccacgcgattacgtccgcgcatagcctggcggcggctttgatcgacaaccacatctattgggcgaatgaattgaatatcgatgtgcgccgtattcattggcgtcgtgttgttgatatgaatgatcgtgcgctgcgcgcaattaaccagagcttgggaggcgtggctaatggtttcccgcgtgaagatggtttcgatatcaccgtggcgagcgaagttatggccgttttctgtctggcgaagaacctggcggacctggaggaacgtctgggccgtatcgtgattgccgagacccgtgaccgtaaaccagttaccttggcggacgtcaaagctaccggtgcaatgaccgtcctgctgaaggacgcgctgcagccgaatctggtacagaccttggagggcaacccggcgctgatccacggcggtccgtttgcgaacattgcgcacggttgtaactcggtgattgcgacgagaactggtctgcgcttggcggactacaccgtgactgaggcaggcttcggcgccgacttaggtgcagaaaagtttatcgacatcaagtgccgtcaaaccggtctcaagccgagcgcggttgttattgtggctaccattcgtgcactgaagatgcatggtggtgttaacaaaaaagacctgcaagcagagaacctggatgctctggagaaaggtttcgccaacttggagcgccacgtgaacaacgtgcgttcctttggtttaccggtcgttgtcggtgttaatcattttttccaggataccgatgcggaacatgcccgtttgaaggagctttgccgtgatagacttcaagtggaagccatcacctgtaaacattgggcagagggcggggctggcgcagaggcactcgcccaagccgtggtgaaattggcggagggcgaacaaaaaccgctgacctttgcgtacgaaaccgagacgaaaatcactgacaaaattaaggccattgcgaccaaactgtacggcgctgcggacatccagattgaaagcaaagcagcaacgaaactggcgggctttgaaaaggatggttatggcggcctgccggtgtgcatggcaaaaacccagtattcgttctccaccgatccgacgctgatgggtgcgccaagcggtcatctggtttccgtccgtgacgtacgcttatctgccggcgcgggcttcgtggttgtcatctgcggtgagatcatgacgatgccgggtttaccgaaggtgcctgcagcggacaccattcgcctcgacgctaatggtcagatcgacggcctgttttaacaattgaaagaggagaaatactagatggctggaaatgaaactatagagacatttttggatggtctcgcgagcagcgccccgacgccaggtggcggtggcgcggctgcgatcagcggtgctatgggcgcggcgttggttagcatggtttgtaatttgaccattggtaaaaagaagtatgtcgaggtggaagcggatctgaagcaggttcttgagaagtccgagggcttgagacgtaccctgactggtatgattgcagacgacgtcgaggcctttgatgcagtgatgggtgcttacggcttaccgaaaaacacggacgaagaaaaagcagcgcgtgcagctaagatccaagaggctctgaagaccgcaaccgacgtgccgctggcgtgctgccgcgtgtgccgtgaagttattgatctggctgaaatcgtggccgagaagggtaatctgaacgtgatctccgatgccggtgttgcagttctgtctgcgtacgcaggcctgcgcagcgcggcgctgaatgtatacgtgaacgccaaaggcctggacgaccgtgcgttcgcggaggagcgcctgaaagaactggagggcttgctggcggaagcgggtgcgctgaacgaacgtatttatgaaaccgttaaatcgaaagtcaactaactcgagagaggagaaatcaaagatgtcaaaaaagttactattccaatttgatactgacgcgacgccgagcgttttcgatgttgtggtcggatacgacggcggtgcggaccacattacgggttacggcaacgtcaccccggataatgttggtgcgtatgttgatggcaccatttacacccgtggtggtaaggagaaacagtccaccgcgattttcgtgggtggcggtgatatggcagccggcgaacgtgttttcgaggcagtgaaaaagcgcttctttggtccgtttagagttagctgtatgctggacagcaatggttctaacaccaccgctgcagcgggcgttgcattggttgtgaaggccgccggtggtagtgttaagggcaagaaggcggtggtactggcgggcaccggcccagttggtatgcgtagcgcagctttgctggctggcgagggtgccgaggtggtgctttgcggtcgtaaactggataaagcgcaagctgctgcggactccgtgaacaaacgcttcaaagtcaacgttaccgcggccgagacagcggacgacgcgagccgtgctgaagcagtgaagggtgcccactttgtgttcaccgctggcgcgattggcctggaactgctgccgcaggcggcgtggcagaatgaatcttcgattgaaatcgtcgcggattataacgcgcaaccgccgctgggtatcggtggtatcgatgcgacggacaagggtaaggaatatggcggcaagcgcgcatttggcgcactcggcatcggcggtctgaaactgaaactgcatcgtgcgtgcatcgccaagttatttgagagcagcgaaggtgtgttcgacgcggaagaaatctacaaattggctaaagagatggcataagatct

SEQ ID NO: 3 - DNA, 1246 bp, synthetic construct
  source 1..1246: mol_type = other DNA
catatgaaaatcggcatcattggtgcaatggaagaagaagttacgctgctgcgtgacaaaatcgaaaaccgtcaaactatcagtctcggcggttgcgaaatctataccggccaactgaatggaaccgaggttgcgcttctgaaatcgggcatcggtaaagtcgctgcggcgctgggtgccactttgctgttggaacactgcaagccagatgtgattattaacaccggttctgccggtggcctggcaccaacgttgaaagtgggcgatatcgttgtctcggacgaagcacgttatcacgacgcggatgtcacggcatttggttatgaatacggtcagttaccaggctgtccggcaggctttaaagctgacgataaactgatcgctgccgctgaggcctgcattgccgaactgaatcttaacgctgtacgtggcctgattgttagcggcgacgctttcatcaacggttctgttggtctggcgaaaatccgccacaacttcccacaggccattgctgtagagatggaagcgacggcaatcgcccatgtctgccacaatttcaacgtcccgtttgttgtcgtacgcgccatctccgacgtggccgatcaacagtctcatcttagcttcgatgagttcctggctgttgccgctaaacagtccagcctgatggttgagtcactggtgcagaaacttgcacatggctaacaattgaaagaggagaaataccatatgccgttgttagatagcttcacagtcgatcatacccggatggaagcgcctgcagttcgggtggcgaaaacaatgaacaccccgcatggcgacgcaatcaccgtgttcgatctgcgcttctgcgtgccgaacaaagaagtgatgccagaaagagggatccataccctggagcacctgtttgctggttttatgcgtaaccatcttaacggtaatggtgtagagattatcgatatctcgccaatgggctgccgcaccggtttttatatgagtctgattggtacgccagatgagcagcgtgttgctgatgcctggaaagcggcaatggaagacgtgctgaaagtgcaggatcagaatcagatcccggaactgaacgtctaccagtgtggcacttaccagatgcactcgttgcaggaagcgcaggatattgcgcgtagcattctggaacgtgacgtacgcatcaacagcaacgaagaactggcactgccgaaagagaagttgcaggaactgcacatctagatct

SEQ ID NO: 4 - DNA, 1418 bp, synthetic construct
  source 1..1418: mol_type = other DNA
catatgtcagcagtaatgacacccgctggatttacggactacaaagttgcagatattaccctcgcggcttggggtcgtagagaactgatcatagcagagtccgaaatgccggcgctgatgggcctgcgtcgcaaatacgccggtcaacagccgctgaagggtgcgaaaatcctgggctgcattcacatgaccattcagactggcgtactgatcgaaacgctagtggccttgggggcggaggtgcgttggtccagctgcaatatctttagcacccaagatcaggcggcggcggctattgcggcagctggcatcccggtttttgcatggaaaggtgaaaccgaggaagaatatgaatggtgtattgagcagaccatcctgaaagatggccaaccgtgggatgcaaatatggttctggacgacggcggtgatctgaccgagatccttcacaagaagtacccgcagatgttggaacgcattcacggtatcaccgaggagaccaccactggcgtgcatcgtctgctggacatgctgaagaacggtactttgaaggtgccggcgatcaatgttaacgacagcgtcaccaaatcgaaaaatgacaacaaatacggctgccgtcacagcttgaatgacgcaattaaacgtggtactgaccatctgttatctggtaagcaagctttagttattggttatggtgatgttggtaaaggttcctctcagagcctccgccaggagggcatgattgttaaggtggcggaagtcgatccgatctgtgcaatgcaagcgtgcatggatggattcgaagtggtgtcgccgtataaaaacggcatcaacgacgggacggaggctagcattgacgctgctctgctgggcaagatcgacttgatcgtgaccacgacgggtaacgtgaatgtgtgtgatgcgaacatgctgaaagccctgaagaagcgggcagttgtgtgcaacatcggccactttgacaatgagatcgataccgcatttatgcgtaagaactgggcgtgggaagaggtcaaaccgcaagtgcacaaaatccatcgcacgggtaaggacggcttcgacgcgcataacgacgattacctgattctgctggcggagggtcgtttagtgaacctgggtaacgcaaccggtcatccgagccgtattatggacggtagctttgccaaccaggttttagcgcagattcacctcttcgagcaaaaatatgcggatctgccagcggcggagaaagccaagcgcttgtcagttgaagttttgcctaagaagctggatgaagaggttgccctggaaatggttaagggcttcggtggcgtagttacccagctgaccccgaaacaagcggagtacatcggcgtcagcgtcgaaggtccattcaagccggatacctatcgttactaagatct

SEQ ID NO: 5 - DNA, 1076 bp, synthetic construct
  source 1..1076: mol_type = other DNA
catatgacagcaactcacaggtcagctaattattccaagccggcgcaactggatatgccgggcttagcgaacttgctgtttggtcatgctgcgttccagtacctgcaagcggcgtgcgaattgaatgtgctggagacagtgcgcaccctgcctgatccgaccaaagagaagctgcgtgaagcgctaggcttagaggagcgtgcagcggatattctgcttcttggcgttaccgcattgggtctgttggttaaagacaacggtgtgtaccacgtggccgatgttgtgcgtgagctgatggataccgatgattggcagagattcaaggacaccgtcgctttcgaacattatatcgtgtacgagggtcagattgacttcaccgaatccctgcaaaaaaacaccaatgttggcttgcgccgttttccgggcgaagggcgcgatatctaccaccgtctgcaccaaaacccgaagctggagaaggtcttttatcgttatatgcgtagctggtcggaactggccaacaaagacctcgtccagcatctggacctgagcaccacccaccgcctgttggacgcgggtggcggtgacgctgtgaacgcactcgcgttggcgcaggcgaacccgaagttagaggtgacggttctggacatcagtcattccattccggttacgcaaagcaaaatcgacgagtctggtctgggtgatcgtgtaaatgcgaaggcgttggacatcctgcacgaaccgttcccaagcggttatgactgtattctgttcgctcaccagctggttatttggacgctggaagagaacacccacatgctgaaaaaagcctatgacgcactgccggaaggtggccgtgtcgtgatttttaattctatgagcaatgatgagggcgatggtccgatcgtggcagcgttggacagcgtttacttcgcgtgcctgccggcagaaggcggaatgatttacgcttgggaacagtacgagcgctgcctggctgaagttggctttaagcatccgcaacgtatccatgttccgggttggactccacatggtattatcatcgcccacaaataagatct

SEQ ID NO: 6 - DNA, 1554 bp, synthetic construct
  source 1..1554: mol_type = other DNA
agatctagaggagaaaactagtatgcctgatatgaagctttttgctggtaacgccaccccggaactagcacaacgtattgccaaccgcctgtacacttcactcggcgacgccgctgtaggtcgctttagcgatggcgaagtcagcgtacaaattaatgaaaatgtacgcggtggtgatattttcatcatccagtccacttgtgcccctactaacgacaacctgatggaattagtcgttatggttgatgccctgcgtcgtgcttccgcaggtcgtatcaccgctgttatcccctactttggctatgcgcgccaggaccgtcgcgtccgttccgctcgtgtaccaatcactgcgaaagtggttgcagacttcctctccagcgtcggtgttgaccgtgtgctgacagtggatctgcacgctgaacagattcagggtttcttcgacgttccggttgataacgtatttggtagcccgatcctgctggaagacatgctgcagctgaatctggataacccaattgtggtttctccggacatcggcggcgttgtgcgtgcccgcgctatcgctaagctgctgaacgataccgatatggcaatcatcgacaaacgtcgtccgcgtgcgaacgtttcacaggtgatgcatatcatcggtgacgttgcaggtcgtgactgcgtactggtcgatgatatgatcgacactggcggtacgctgtgtaaagctgctgaagctctgaaagaacgtggtgctaaacgtgtatttgcgtacgcgactcacccgatcttctctggcaacgcggcgaacaacctgcgtaactctgtaattgatgaagtcgttgtctgcgataccattccgctgagcgatgaaatcaaatcactgccgaacgtgcgtactctgaccctgtcaggtatgctggccgaagcgattcgtcgtatcagcaacgaagaatcgatctctgccatgttcgaacactaaggtaccaaagaggagaaatactagatgaccgcgactgcacagcagcttgagtatctcaaaaatagcatcaaaagcattcaggactacccaaaacccggcattcttttccgcgatgtcaccagcttactggaagacccgaaagcttacgctctcagcatcgacttgctggttgagcgttacaaaaatgcgggcattaccaaagttgtcggcaccgaagcgcgtggcttcttgtttggcgctccggtagctctgggtctgggcgttggctttgtaccggtccgtaaaccgggcaaactgccgcgtgaaaccatcagtgaaacttacgacctggaatacggcaccgatcagctggagatccacgttgatgccatcaaaccgggcgacaaagttctggtggtggacgacctgctggcaaccggcggcactatcgaagcgaccgttaaactgatccgtcgtctgggtggtgaagtggctgacgctgcgttcattatcaacctgttcgatctcggcggcgaacagcgtctcgaaaaacagggcattaccagctacagccttgtcccgttcccgggccattaaggccggcc

SEQ ID NO: 7 - DNA, 1053 bp, synthetic construct
  source 1..1053: mol_type = other DNA
agatctaaagaggagaaatactagatgacagctcccttagttgtactaggaaatccactgttggacttccaagcagatgttacggctgaatacctggcgaagtactctctgaaagaaaacgatgccattttggtggatgcgaagtccggtgatgcaaagatggcgatttttgatgaactgctgcagatgccggaaaccaaactggttgcagggggtgcggctcaaaacaccgctcgcggtgcggcgtatgttctgggcgctggccaagttgtctacttcggctccgttggcaaggacaaatttagtgaacgtttactgaacgagaacgagaaagcaggtgtcaaaagcatgtatcaggttcagaatgacattggtacgggtaagtgcgctgcgcttatcaccggtcataatcgcagcttggtaactgacctgggtgcggcgaacttttttacgcctgaccacctggacaaacattgggatttggtcgaggccgccaagctgttctacatcggcggcttccacctgactgttagcccggacgcgatcgtgaagctcggacaacacgcaaaagagaacagcaaaccgttcgtgctcaattttagcgcaccgtttatcccacatgtttttaaagacgccctggcgcgtgtcctgccgtatgcgaccgtcatcatcgccaacgagagcgaagcggaagcgttctgcgatgctttccagctggactgtgcgaacaccgatttggaagccatcgcgcaacgtattgttaaggactctccggttgagaaaaccgtgattttcacccacggcgtggagccgaccgtggtggtgagctcgaaaggcacctcgacctatccggtgaagccgttggacagctcaaaaatcgtggataccaatggtgcaggcgacgctttcgccggcggttttatggctggcctgaccaagggtgaggatttggagacatctattgatatgggtcagtggctggcagcgctgagcattcaggaggttggtccgtcctacccgtccgaaaagatcagctacagcaagtaacaattg

SEQ ID NO: 8 - DNA, 3405 bp, synthetic construct
  source 1..3405: mol_type = other DNA
ccatggcagcgacagctgctctaaggtcaggagacacccgtgctcaaaccgcggcggcgttcccgccacctccggtgacggctcgccccatcgaccgcgctgcgtggatcgccgcgttccgcttcgtgcgttccgaaactgagcgccgtgctgctccgttgtctgctgaagatcagcaggttcagagcatggcggacgcaagcccgacaaaatggcaccgtgcgcacgtgacgtggttcttcgagcagttcctgctgcgtgagcacctgccgggttacgcaatttatgacgaacgtctgcactacctgtttaactcctattacgtggctgcgggcccgcgtcagccgcgtatccagcgtggcatgattacccgtccgacgatggcggaggtgactgcgtaccgtgcacacgtcgatcgtgccgtcgagtcgctgctggggcaagcggcggacggcgcgttggaagcggtgctgccgatcttggagatcggcttatatcatgaacaacaacatcaagaactgttgttgaccgatatcctccacgccttcgcccaaaacccgctaggcccagtctatgacgcggagtggcgtttcccggcagtggctggccagggtggccaggctccgctggcgagaggtattgcatggattggtcacgagggtgatggtttttcttttgacaacgagtccccgcgtcatgaggccctcattctgcctggacgtatcgataaagcgttggttaccaatcgcgactggctgggctttatggaagccggtggttacgccaagccggaactgtggctgtcagacggctggtatgcgggtcaagcggagggttgggaggcaccgggctactggcgtcgtgatggtgaaggctgggcaaccatgaccctgggtggtgttcgtccggtagagctggatgcaccggtcacgcatattagctactatgaggccgatgcctacgcgcgctgggcaggccgtaccctgccgacggaatttgagtgggaagttgcagctcgcgacggcgcacttccggatgcatttggtcttgtttggcaatggaccagaagcgcgtacgttgcgtacccgggttaccggccactgccgggtgcgctgggcgaatataacggcaagtttatggttagccagttcgtgctgcgtggtagcagcgttgcgaccccggaaggccacgcacgcttgccgtatcgtaattttttttatccgcatcagcgttggcagttcaccggtttgcgcctggcggacgtggcctaaacgcgtagaggagaaatacatcatgacattgtcactagctaattatttagcagcggactctgccgcggaggcgctgcgtcgcgatgttcgtgcgggcttgactgcggctccgaagagcctgccaccaaagtggttttacgacgctgtgggctccgatttgtttgaccagattacccgtctgccggaatattacccgacccgtaccgaagctcaaatcctgcgtaccagaagcgcagagatcatcgcggcggctggtgcagataccctcgtggagctgggcagcggtacgagcgaaaaaacccgcatgctgctggacgctatgcgagacgctgagttgttgcgtcgttttatcccgtttgacgtggatgccggggtgctgcgctctgcgggagcggcgattggcgcagagtacccgggtattgagatcgatgcggtctgtggtgatttcgaagagcacctgggcaaaatcccgcatgttggtcgtcgtttagtagtctttcttggcagtaccattggtaatctgactccggcaccgcgtgcagagttcctgagcaccttggcggacaccctgcagccgggtgactccttgctgttgggtaccgacctggttaaagataccggtcgcctggttcgcgcgtatgatgatgcggcgggcgttaccgcggcgttcaaccgcaacgttctggcggtggtgaaccgtgaattgtcggctgacttcgacttagacgcgttcgagcacgtggccaaatggaacagcgacgaagaacgtattgagatgtggctgcgtgcgcgtacggcccaacacgtgcgtgttgcagcgctggatctggaagtggacttcgcagctggtgaagagatgctcacggaagttagctgcaagtttcgtccggaaaatgttgttgcagagctggctgaggcgggcctgcgccagacccattggtggaccgatccggcaggcgacttcggtctctccctggccgtccgctaaggatccaaagaggagaaaactagtatgatgctagctcagcaatggagggatgcacgtccgaaagtggcgggtctgcacctggactccggtgcatgcagccgtcaaagctttgcggtcatcgacgccacgactgcgcacgcacgccacgaagcagaggtgggcggttatgttgctgcggaggcggctaccccggcgctcgacgctggccgtgcggcggtggcctctctgattggtttcgccgcttccgatgtggtgtacaccagcggtagcaaccacgcgattgatctgctgctgtcttcctggccgggtaagcgcaccctggcgtgtctgccgggtgaatatggccccaacctgagcgcaatggcagcgaatggtttccaggttcgtgcactgccggtggacgacgacggtcgcgtgctggtagacgaagccagccacgagctcagtgcccacccggttgcgttggtgcatcttaccgcgctcgcgtcccatcgtggtatcgcccaaccggcggcggaattggtcgaggcgtgccataacgccggtattccggttgtgatcgatgctgctcaggcacttggtcatctggactgtaatgttggcgctgatgccgtttacagctcgtcccgtaaatggctggcgggtccgcgtggcgttggcgtgctggcggttcgcccggaattggcggagcgcctgcagccgagaatcccaccgtcagattggcctattccgatgagcgttttggagaagctggagttaggtgaacacaacgcagcggcgcgtgtgggcttcagcgttgcggtaggcgagcacctggcggctggtccgaccgccgtgcgcgagcgtttggcggaggtcggccgcctgagccgtcaagttctggcagaagtggacggctggcgtgtggttgaaccggtggaccagccgacggcaatcaccaccttggagagcaccgatggcgccgatccggcttctgttcgtagctggctgatcgcggaacgtggcattgttactacggcctgcgaactggcgcgtgcaccgtttgaaatgcgtaccccggtgttgcgcatcagcccgcatgttgatgttaccgtagacgagctggaacagtttgcagcggctctgagagaagcgccataagaattc

SEQ ID NO: 9 - DNA, 1045 bp, synthetic construct
  source 1..1045: mol_type = other DNA
ccatgggaagttcagaagatcaagcttataggttgctgaacgattacgcaaatggttttatggtcagccaagttctgtttgcggcgtgtgaacttggcgtattcgacctgttagccgaagcaccgggcccgctcgacgtggcagcggtggctgcgggtgttagagcgagcgcgcatggtactgagctgttgttggacatctgcgtttctctgaagctgctgaaggtggaaacccgaggtggcaaggcgttctatcgtaacaccgagctgtctagtgattacctgacgaccgtgtccccgaccagccagtgttccatgctcaagtacatgggtcgcacgagctatcgttgctggggtcatctggctgacgctgtccgtgaaggtcgcaaccagtatctggaaacctttggtgtgccggcagaggagctcttcaccgcgatctaccgcagcgaaggtgaacgtctccaattcatgcaggctctgcaagaggtttggtccgttaatggccgtagcgttctgactgccttcgacctatccgtgttcccgctgatgtgcgatctgggcggcggagccggtgcgctggcgaaagagtgcatgagcttgtacccaggctgcaaaatcacggtattcgacatcccggaagtcgtgtggaccgcgaagcagcacttcagctttcaagaagaggagcagattgatttccaagagggtgacttctttaaagatccgttaccggaggcagacctgtacattctggcccgtgttctgcacgattgggaagacggcaagtgcagccacctgttggagcgcatttaccacacctgtaaaccgggtggcggtattctggtgattgaaagccttctggacgaagatcgtcgtggcccattgctgacgcagctgtatagcctgaacatgttggttcagaccgagggccaggagcgcaccccgacccattatcacatgctgttgtcttcggctggttttcgtgactttcaatttaaaaaaaccggtgcgatctatgatgcgatcctcgctcgtaaataagatct

SEQ ID NO: 10 - DNA, 1182 bp, synthetic construct
  source 1..1182: mol_type = other DNA
catatgacacacctaaacatagctaatagggtagacagcttcttcatcccgtgcgtcaccttgtttggtccgggttgtgttcgtgagacaggtgtgcgcgcacgtagcttgggcgctcgcaaggctctgatcgtcactgacgccggcctccacaaaatgggtttgtcggaagttgttgcgggccacattcgtgaggcgggtctgcaggcagttatcttcccgggtgcggagccgaatccgaccgatgttaatgttcacgacggcgtgaagctgtttgaaagagaggaatgcgattttatcgtgtccctgggaggtggctcctctcatgactgcgcgaaaggtattggcttggttaccgcgggcggaggccacatacgcgattacgaaggtattgacaaaagcacggttccgatgactccgttgatcagcattaacacgacggcaggaaccgcggcggagatgacccgtttctgcatcatcacgaacagcagcaatcatgtgaagatggtcattgtggattggcgttgtaccccgctaattgcgattgacgacccgagcctaatggtcgccatgccgccggccctgactgcggctaccggtatggatgcgctgacccatgcgatcgaggcctacgtgtccaccgcggcgacgccaatcaccgacgcctgcgctgagaaagcgatcgtgctgatcgcagagtggctgccgaaagctgtggccaatggcgattctatggaagcgcgtgcagctatgtgctacgcgcaatacctggctggcatggcatttaacaacgcgtcgctgggttatgttcacgcaatggcgcaccagctgggcggcttttataacctgccacatggtgtgtgtaatgcgatcctcttgccgcacgttagcgagttcaacctgatcgccgcgccagaacgttatgctcgcattgcagagctgctgggtgaaaacattggtggccttagcgcccacgatgcggccaaggcggcagtgtcagccatccgtaccctgtctaccagcatcggtattccggcaggcctggctggtttaggggtcaaggccgacgaccatgaagttatggcgtccaacgcacagaaagatgcgtgcatgctgaccaacccgcgtaaggcaaccttagctcaagtaatggctattttcgcggcggcgatgtaagacgtc